European Patent Application EP 4 796 630 A2, published August 26, 2026. Title: A cell-based method for determining an activity of botulinum toxin. Applicant: Hugel Inc. Application EP, filed January 10, 2019. The sequence listing filed with the application follows.

SEQUENCE LISTING (90 sequences)

SEQ ID NO: 1 - protein, 13 aa, clostridium botulinum
MAEDADMRNELEE

SEQ ID NO: 2 - protein, 13 aa, clostridium botulinum
MAEDADMRNELEE

SEQ ID NO: 3 - protein, 20 aa, clostridium botulinum
DQLADESLESTRRMLQLVEE

SEQ ID NO: 4 - protein, 20 aa, clostridium botulinum
DEQGEQLERIEEGMDQINKD

SEQ ID NO: 5 - protein, 15 aa, clostridium botulinum
DEREQMAISGGFIRR

SEQ ID NO: 6 - protein, 15 aa, clostridium botulinum
EIDTQNRQIDRIMEK

SEQ ID NO: 7 - protein, 15 aa, clostridium botulinum
RIMEKADSNKTRIDE

SEQ ID NO: 8 - protein, 18 aa, clostridium botulinum
RIMEKADSNKTRIDEANQ

SEQ ID NO: 9 - protein, 12 aa, clostridium botulinum
DSNKTRIDEANQ

SEQ ID NO: 10 - protein, 13 aa, clostridium botulinum
KTRIDEANQPATK

SEQ ID NO: 11 - protein, 9 aa, synthetic construct
  REGION 1..9: note = antibody CDR of clostridium botulinum
GYSITSGYY

SEQ ID NO: 12 - protein, 8 aa, synthetic construct
  REGION 1..8: note = antibody CDR of clostridium botulinum
GYTFTDYN

SEQ ID NO: 13 - protein, 8 aa, synthetic construct
  REGION 1..8: note = antibody CDR of clostridium botulinum
GYTFTNYG

SEQ ID NO: 14 - protein, 7 aa, synthetic construct
  REGION 1..7: note = antibody CDR of clostridium botulinum
IRYDGSN

SEQ ID NO: 15 - protein, 8 aa, synthetic construct
  REGION 1..8: note = antibody CDR of clostridium botulinum
IYPYNGDT

SEQ ID NO: 16 - protein, 8 aa, synthetic construct
  REGION 1..8: note = antibody CDR of clostridium botulinum
INTYTGEP

SEQ ID NO: 17 - protein, 12 aa, synthetic construct
  REGION 1..12: note = antibody CDR of clostridium botulinum
ARDRDSSYYFDY

SEQ ID NO: 18 - protein, 6 aa, synthetic construct
  REGION 1..6: note = antibody CDR of clostridium botulinum
VRSGDY

SEQ ID NO: 19 - protein, 7 aa, synthetic construct
  REGION 1..7: note = antibody CDR of clostridium botulinum
ARGYYDY

SEQ ID NO: 20 - protein, 6 aa, synthetic construct
  REGION 1..6: note = antibody CDR of clostridium botulinum
DHINNW

SEQ ID NO: 21 - protein, 11 aa, synthetic construct
  REGION 1..11: note = antibody CDR of clostridium botulinum
QSLLDSNGKTY

SEQ ID NO: 22 - protein, 11 aa, synthetic construct
  REGION 1..11: note = antibody CDR of clostridium botulinum
QSLLDSDGKTY

SEQ ID NO: 23-24 - skipped (2 entries)

SEQ ID NO: 25 - protein, 9 aa, synthetic construct
  REGION 1..9: note = antibody CDR of clostridium botulinum
QQYWSAPPT

SEQ ID NO: 26 - protein, 9 aa, synthetic construct
  REGION 1..9: note = antibody CDR of clostridium botulinum
WQGTLFPYT

SEQ ID NO: 27 - protein, 9 aa, synthetic construct
  REGION 1..9: note = antibody CDR of clostridium botulinum
WQGTHFPRT

SEQ ID NO: 28 - protein, 9 aa, synthetic construct
  REGION 1..9: note = antibody CDR of clostridium botulinum
GYSITSDYA

SEQ ID NO: 29 - protein, 8 aa, synthetic construct
  REGION 1..8: note = antibody CDR of clostridium botulinum
GFTFNTNA

SEQ ID NO: 30 - protein, 8 aa, synthetic construct
  REGION 1..8: note = antibody CDR of clostridium botulinum
GYTFTNYT

SEQ ID NO: 31 - protein, 8 aa, synthetic construct
  REGION 1..8: note = antibody CDR of clostridium botulinum
GYTFNTYA

SEQ ID NO: 32 - protein, 8 aa, synthetic construct
  REGION 1..8: note = antibody CDR of clostridium botulinum
GFTFSNYG

SEQ ID NO: 33 - protein, 8 aa, synthetic construct
  REGION 1..8: note = antibody CDR of clostridium botulinum
GFTFNTYA

SEQ ID NO: 34 - protein, 7 aa, synthetic construct
  REGION 1..7: note = antibody CDR of clostridium botulinum
ISYSVGT

SEQ ID NO: 35 - protein, 10 aa, synthetic construct
  REGION 1..10: note = antibody CDR of clostridium botulinum
IRSKSNNYAT

SEQ ID NO: 36 - protein, 10 aa, synthetic construct
  REGION 1..10: note = antibody CDR of clostridium botulinum
IRSKSDNYAT

SEQ ID NO: 37 - protein, 8 aa, synthetic construct
  REGION 1..8: note = antibody CDR of clostridium botulinum
INPSSDYT

SEQ ID NO: 38 - protein, 10 aa, synthetic construct
  REGION 1..10: note = antibody CDR of clostridium botulinum
IRSKSNNYTT

SEQ ID NO: 39 - protein, 8 aa, synthetic construct
  REGION 1..8: note = antibody CDR of clostridium botulinum
INSNGGTT

SEQ ID NO: 40 - protein, 10 aa, synthetic construct
  REGION 1..10: note = antibody CDR of clostridium botulinum
ARKGEYGFAY

SEQ ID NO: 41 - protein, 11 aa, synthetic construct
  REGION 1..11: note = antibody CDR of clostridium botulinum
VYGRSYGGLSY

SEQ ID NO: 42 - protein, 11 aa, synthetic construct
  REGION 1..11: note = antibody CDR of clostridium botulinum
VYGRSYGGLGY

SEQ ID NO: 43 - protein, 13 aa, synthetic construct
  REGION 1..13: note = antibody CDR of clostridium botulinum
VRQVTTAVGGFAY

SEQ ID NO: 44 - protein, 16 aa, synthetic construct
  REGION 1..16: note = antibody CDR of clostridium botulinum
ARRIFYNGRTYAAMDY

SEQ ID NO: 45 - protein, 17 aa, synthetic construct
  REGION 1..17: note = antibody CDR of clostridium botulinum
VGQILYYYVGSPAWFAY

SEQ ID NO: 46 - protein, 9 aa, synthetic construct
  REGION 1..9: note = antibody CDR of clostridium botulinum
ARDRDAMDY

SEQ ID NO: 47 - protein, 10 aa, synthetic construct
  REGION 1..10: note = antibody CDR of clostridium botulinum
KSVSTSGYSY

SEQ ID NO: 48 - protein, 10 aa, synthetic construct
  REGION 1..10: note = antibody CDR of clostridium botulinum
KSVSSSGYSY

SEQ ID NO: 49 - protein, 11 aa, synthetic construct
  REGION 1..11: note = antibody CDR of clostridium botulinum
QSIVNSHGNTY

SEQ ID NO: 50-51 - skipped (2 entries)

SEQ ID NO: 52 - protein, 9 aa, synthetic construct
  REGION 1..9: note = antibody CDR of clostridium botulinum
QHSRELPLT

SEQ ID NO: 53 - protein, 9 aa, synthetic construct
  REGION 1..9: note = antibody CDR of clostridium botulinum
QHSRELPWT

SEQ ID NO: 54 - protein, 9 aa, synthetic construct
  REGION 1..9: note = antibody CDR of clostridium botulinum
FQGSHVPWT

SEQ ID NO: 55 - protein, 8 aa, synthetic construct
  REGION 1..8: note = antibody CDR of clostridium botulinum
GFTFSNYG

SEQ ID NO: 56 - protein, 8 aa, synthetic construct
  REGION 1..8: note = antibody CDR of clostridium botulinum
GINIKDYY

SEQ ID NO: 57 - protein, 8 aa, synthetic construct
  REGION 1..8: note = antibody CDR of clostridium botulinum
ISSGGSYT

SEQ ID NO: 58 - protein, 8 aa, synthetic construct
  REGION 1..8: note = antibody CDR of clostridium botulinum
IDPGNGDA

SEQ ID NO: 59 - protein, 13 aa, synthetic construct
  REGION 1..13: note = antibody CDR of clostridium botulinum
ARHEGGGNPYFDY

SEQ ID NO: 60 - protein, 5 aa, synthetic construct
  REGION 1..5: note = antibody CDR of clostridium botulinum
NEIAY

SEQ ID NO: 61 - protein, 11 aa, synthetic construct
  REGION 1..11: note = antibody CDR of clostridium botulinum
QSLVHSNGNTY

SEQ ID NO: 62 - protein, 11 aa, synthetic construct
  REGION 1..11: note = antibody CDR of clostridium botulinum
QSLLDSDGKTY

SEQ ID NO: 63-64 - skipped (2 entries)

SEQ ID NO: 65 - protein, 9 aa, synthetic construct
  REGION 1..9: note = antibody CDR of clostridium botulinum
SQNTLVPWT

SEQ ID NO: 66 - protein, 9 aa, synthetic construct
  REGION 1..9: note = antibody CDR of clostridium botulinum
WQGTHFPFT

SEQ ID NO: 67 - protein, 120 aa, synthetic construct
  REGION 1..120: note = antibody of clostridium botulinum
EVKLVESGGGLVKPGGSLKLSCAASGFTFSNYGMSWVRQTPEKRLEWVATISSGGSYTYYPDSVKGRFTISRDNAKNTLYLQMSSLRSEDTAMYYCARHEGGGNPYFDYWGQGTTLTVSS

SEQ ID NO: 68 - protein, 112 aa, synthetic construct
  REGION 1..112: note = antibody of clostridium botulinum
DVLMTQTPLSLPVSLGDQASISCRSSQSLVHSNGNTYLHWYLQKPGQSPKLLIYKVSNRFSGVPDRFSGSGSGTDFTLKISRVEAEDLGVYFCSQNTLVPWTFGGGTKLEIK

SEQ ID NO: 69 - protein, 112 aa, synthetic construct
  REGION 1..112: note = antibody of clostridium botulinum
EVQLQQSGAELVRPGASVKLSCTASGINIKDYYMHWMKQRPEQDLEWIGWIDPGNGDAEYAPKFQGKATMTADTSSNTAYLQLSSLTSEDTAVYYCNEIAYWGQGTLVTVSA

SEQ ID NO: 70 - protein, 112 aa, synthetic construct
  REGION 1..112: note = antibody of clostridium botulinum
DIVMTQSPLTLSVTIGQPASISCKSSQSLLDSDGKTYLNWLLQRPGQSPKRLIYLVSKLDSGVPDRFTGSGSGTDFTLKISRVEAEDLGVYYCWQGTHFPFTFGSGTKLEIK

SEQ ID NO: 71 - protein, 117 aa, synthetic construct
  REGION 1..117: note = antibody of clostridium botulinum
DVKLQESGPGLVKPSQSLSLTCTVTGYSITSDYAWNWIRQFPGNKLEWMGYISYSVGTRYNPSLKSRISITRDTSKNQFFLLLKSVTNEDTATYFCARKGEYGFAYWGQGTLVTVSA

SEQ ID NO: 72 - protein, 111 aa, synthetic construct
  REGION 1..111: note = antibody of clostridium botulinum
DIVMTQSPASLAVSLGQRATISCRASKSVSTSGYSYMHWYQQKPGQPPKLLIYLASNLESGVPARFSGSGSGTDFTLNIHPVEEEDAATYYCQHSRELPLTFGAGTKLELK

SEQ ID NO: 73 - protein, 120 aa, synthetic construct
  REGION 1..120: note = antibody of clostridium botulinum
QVQLVETGGGLVQPKGSLKLSCAASGFTFNTNAMNWVRQAPGKGLEWVARIRSKSNNYATYYADSVKDRFTISRDDSQSLLYLQMNNLKTEDTAMYYCVYGRSYGGLSYWGQGTLVTVSA

SEQ ID NO: 74 - protein, 111 aa, synthetic construct
  REGION 1..111: note = antibody of clostridium botulinum
DIVMTQSPASLAVSLGQRATISCRASKSVSSSGYSYMHWYQQKPGQPPKLLIYLASNLESGVPARFSGSGSGTDFTLNIHPVEEEDAATYYCQHSRELPLTFGAGTKLELK

SEQ ID NO: 75 - protein, 120 aa, synthetic construct
  REGION 1..120: note = antibody of clostridium botulinum
EVKLVESGGGLVQPKGSLKLSCAASGFTFNTNAMNWVRQAPGKGLEWVARIRSKSDNYATYYADSVKDRFTISRDDSPSMLYLQMNNLKTEDTAMYYCVYGRSYGGLGYWGQGTLVTVSA

SEQ ID NO: 76 - protein, 111 aa, synthetic construct
  REGION 1..111: note = antibody of clostridium botulinum
DIVLTQSPASLAVSLGQRATISCRASKSVSTSGYSYVHWYQQKPGQPPKLLIYLASNLESGVPARFSGSGSGTDFTLNIHPVEEEDAATYYCQHSRELPLTFGAGTKLELK

SEQ ID NO: 77 - protein, 122 aa, synthetic construct
  REGION 1..122: note = antibody of clostridium botulinum
EVKLVESGGGLVQPKGSLKLSCAASGFTFNTYAMNWVRQAPGKGLEWVARIRSKSNNYATYYADSVKDRFTISRDDSQSMLYLQMNNLKTEDTAMYYCVRQVTTAVGGFAYWGQGTLVTVSE

SEQ ID NO: 78 - protein, 111 aa, synthetic construct
  REGION 1..111: note = antibody of clostridium botulinum
DIVMTQSPASLAVSLGQRTTISCRASKSVSSSGYSYMHWYQQKPGQPPKLLIYLASNLESGVPARFSGSGSGTDFTLNIHPVEEEDAATYYCQHSRELPLTFGAGTKLELR

SEQ ID NO: 79 - protein, 123 aa, synthetic construct
  REGION 1..123: note = antibody of clostridium botulinum
EVQLQQSGAELARPGASVQMSCKAFGYTFTNYTMHWVRQRPGQGLEWIGFINPSSDYTNYNQKFKDKATLSADKSSSTAYMQLSSLTSEDSAVYYCARRIFYNGRTYAAMDYWGQGTSVTVSS

SEQ ID NO: 80 - protein, 111 aa, synthetic construct; identical to SEQ ID NO: 74
  REGION 1..111: note = antibody of clostridium botulinum

SEQ ID NO: 81 - protein, 126 aa, synthetic construct
  REGION 1..126: note = antibody of clostridium botulinum
EVKLVESGGGLVQPKGSLKLSCAASGYTFNTYAMNWVRQAPGKGLEWVARIRSKSNNYTTYYADSVKDRFTISRDDSQSMLYLQINNLKTEDTAMYYCVGQILYYYVGSPAWFAYWGQGTLVTVSA

SEQ ID NO: 82 - protein, 111 aa, synthetic construct
  REGION 1..111: note = antibody of clostridium botulinum
DIVMTQSPASLAVSLGQRATISCRASKSVSTSGYSYMHWYQQKPGQPPKLLIFLASNLESGVPARFSGSGSGTDFTLNIHPVEEEDAATYYCQHSRELPWTFGGGTKLEIK

SEQ ID NO: 83 - protein, 119 aa, synthetic construct
  REGION 1..119: note = antibody of clostridium botulinum
DVKLQESGPGLVKPSQSLSLTCSVTGYSITSGYYWNWIRQFPGNKLEWMGYIRYDGSNNYNPSLKNRISITRDTSKNQFFLKLNSVTTEDTASYYCARDRDSSYYFDYWGQGTALTVSS

SEQ ID NO: 84 - protein, 107 aa, synthetic construct
  REGION 1..107: note = antibody of clostridium botulinum
DIVMTQSSSYLSVSLGGRVTITCKASDHINNWLAWYQQKPGNAPRLLISDTTSLETGVPSRFSGSGSGKDYTLSITSLQTEDVATYYCQQYWSAPPTFGGGTKLEIK

SEQ ID NO: 85 - protein, 116 aa, synthetic construct
  REGION 1..116: note = antibody of clostridium botulinum
EVQLEESGGGLVQPGGSLKLSCAASGFTFSNYGMSWVRQTPDKRLELVATINSNGGTTYYPDSVKGRFTISRDNAKNTLYLQMSSLKSEDSAMYYCARDRDAMDYWGQGTSVTVSS

SEQ ID NO: 86 - protein, 112 aa, synthetic construct
  REGION 1..112: note = antibody of clostridium botulinum
DVLMTQTPLSLPVSLGDQASISCRSSQSIVNSHGNTYLEWYLQKPGQSPKLLIYKVSNRFSGVPDRFSGSGSGTDFTLKISRVEAEDLGVYYCFQGSHVPWTFGGGTKLEIK

SEQ ID NO: 87 - protein, 113 aa, synthetic construct
  REGION 1..113: note = antibody of clostridium botulinum
EVQLQQSGPELVKPGASVKISCKASGYTFTDYNMHWVKQSHGKSLEWIGYIYPYNGDTGYNQKFKSKATLTVDNSSSTAYMELRSLTSEDSAVYYCVRSGDYWGQGTTLTVSS

SEQ ID NO: 88 - protein, 112 aa, synthetic construct
  REGION 1..112: note = antibody of clostridium botulinum
DVLMTQTPLTLSVTIGQPASISCKSSQSLLDSNGKTYLNWLLQRPGQSPSRLIYLVSKLDSGVPDRFTGSGSGTDFTLKISRVEAEDLGVYYCWQGTLFPYTFGGGTKLEIK

SEQ ID NO: 89 - protein, 114 aa, synthetic construct
  REGION 1..114: note = antibody of clostridium botulinum
QIQLAQSGPELKKPGETVKISCKASGYTFTNYGMSWVKQAPGKGLKWMGWINTYTGEPTYAADFKGRFAFSLETSASTAFLQINNLKNEDTATYFCARGYYDYWGQGTTLTVSS

SEQ ID NO: 90 - protein, 112 aa, synthetic construct
  REGION 1..112: note = antibody of clostridium botulinum
DVLMTQTPLTLSVTIGQPASISCKSSQSLLDSDGKTYLNWLLQRPGQSPKRLIYLVSKLDSGVPDRFTGSGSGTDFTLKISRVEAEDLGVYYCWQGTHFPRTFGGGTKLEIK